European Patent Specification EP 3 650 458 B1, published August 9, 2023. Title: CHEMICALLY ENCODED SPATIALLY ADDRESSED LIBRARY SCREENING PLATFORMS. Applicant: City of Hope Berlin, Jacob Copeland, Gregory Elison, Kathleen Muradyan, Hurik. The sequence listing filed with the application follows.

SEQUENCE LISTING (18 sequences)

SEQ ID NO: 1 - DNA, 18 bp, Artificial Sequence
  Synthetic polynucleotide
  misc_feature (1)..(1): Terminal modified with hexynyl
  misc_feature (18)..(18): Terminal modified with AmMO
aaccacacacacacaacc

SEQ ID NO: 2 - DNA, 18 bp, Artificial Sequence
  Synthetic polynucleotide
  misc_feature (1)..(1): Terminal modified with hexynyl
  misc_feature (18)..(18): Terminal modified with AmMO
aaccacacacaccaaacc

SEQ ID NO: 3 - DNA, 18 bp, Artificial Sequence
  Synthetic polynucleotide
  misc_feature (1)..(1): Terminal modified with hexynyl
  misc_feature (18)..(18): Terminal modified with AmMO
acgaacacacacgtacga

SEQ ID NO: 4 - DNA, 18 bp, Artificial Sequence
  Synthetic polynucleotide
  misc_feature (1)..(1): Terminal modified with hexynyl
  misc_feature (18)..(18): Terminal modified with AmMO
caagacacacacgtcaag

SEQ ID NO: 5 - DNA, 18 bp, Artificial Sequence
  Synthetic polynucleotide
  misc_feature (1)..(1): Terminal modified with hexynyl
  misc_feature (18)..(18): Terminal modified with AmMO
ccttacacacacgtcctt

SEQ ID NO: 6 - DNA, 18 bp, Artificial Sequence
  Synthetic polynucleotide
  misc_feature (1)..(1): Terminal modified with hexynyl
  misc_feature (18)..(18): Terminal modified with AmMO
acgaacacacactgacga

SEQ ID NO: 7 - DNA, 18 bp, Artificial Sequence
  Synthetic polynucleotide
  misc_feature (1)..(1): Terminal modified with hexynyl
  misc_feature (18)..(18): Terminal modified with AmMO
caagacacacactgcaag

SEQ ID NO: 8 - DNA, 18 bp, Artificial Sequence
  Synthetic polynucleotide
  misc_feature (1)..(1): Terminal modified with hexynyl
  misc_feature (18)..(18): Terminal modified with AmMO
ccttacacacactgcctt

SEQ ID NO: 9 - DNA, 18 bp, Artificial Sequence
  Synthetic polynucleotide
  misc_feature (1)..(1): Terminal modified with Cy3
tcgtacgtgtgtgttcgt

SEQ ID NO: 10 - DNA, 18 bp, Artificial Sequence
  Synthetic polynucleotide
  misc_feature (1)..(1): Terminal modified with Cy3
cttgacgtgtgtgtcttg

SEQ ID NO: 11 - DNA, 18 bp, Artificial Sequence
  Synthetic polynucleotide
  misc_feature (1)..(1): Terminal modified with Cy3
aaggacgtgtgtgtaagg

SEQ ID NO: 12 - DNA, 18 bp, Artificial Sequence
  Synthetic polynucleotide
  misc_feature (1)..(1): Terminal modified with Alex647
tcgtcagtgtgtgttcgt

SEQ ID NO: 13 - DNA, 18 bp, Artificial Sequence
  Synthetic polynucleotide
  misc_feature (1)..(1): Terminal modified with 6-FAM
cttgcagtgtgtgtcttg

SEQ ID NO: 14 - DNA, 18 bp, Artificial Sequence
  Synthetic polynucleotide
  misc_feature (1)..(1): Terminal modified with 6-FAM
aaggcagtgtgtgtaagg

SEQ ID NO: 15 - DNA, 18 bp, Artificial Sequence
  Synthetic polynucleotide
  misc_feature (1)..(1): Terminal modified with Cy3
ggttgtgtgtgtgtggtt

SEQ ID NO: 16 - DNA, 18 bp, Artificial Sequence
  Synthetic polynucleotide
  misc_feature (1)..(1): Terminal modified with 6-FAM
ggtttggtgtgtgtggtt

SEQ ID NO: 17 - protein, 9 aa, Artificial Sequence
  Synthetic polypeptide
YPYDVPDYA

SEQ ID NO: 18 - protein, 10 aa, Artificial Sequence
  Synthetic polypeptide
EQKLISEEDL